European Patent Application EP 4 685 155 A1, published January 28, 2026. Title: 抗PD-1与突变IL-2免疫缀合物制剂. Applicant: FORTVITA BIOLOGICS (SINGAPORE) PTE. LTD. The sequence listing filed with the application follows.

SEQUENCE LISTING (25 sequences)

SEQ ID NO: 1 - protein, 153 aa, synthetic construct
MYRMQLLSCIALSLALVTNSAPTSSSTKKTQLQLEHLLLDLQMILNGINNYKNPKLTRMLTFKFYMPKKATELKHLQCLEEELKPLEEVLNLAQSKNFHLRPRDLISNINVIVLELKGSETTFMCEYADETATIVEFLNRWITFCQSIISTLT

SEQ ID NO: 2 - protein, 133 aa, synthetic construct [sequence omitted]

SEQ ID NO: 3 - protein, 133 aa, synthetic construct
APTSSSTKKTQLQLEHLLLDLQMILNGINNYKNPKLTRMLTFKFYMPKKATELKHLQCLEEELKPLEEVLNLAQSKNFHLRPRDLISNINVIVLELKGSETTFMCEYADETATIVEFLNRWITFSQSIISTLT

SEQ ID NO: 4 - protein, 129 aa, synthetic construct
APASSSTKKTQLQLEHLLLDLQMILNGINNYKNPKLTRMLTFKFYMPKKATELKHLQCLEEELKPLEEVLNLAGDASIHDLISRINVIVLELKGSETTFMCEYADETATIVEFLNRWITFSQSIIRTLT

SEQ ID NO: 5 - protein, 10 aa, synthetic construct
GGGGSGGGGS

SEQ ID NO: 6 - protein, 227 aa, synthetic construct
DKTHTCPPCPAPEAAGGPSVFLFPPKPKDTLMISRTPEVTCVVVDVSHEDPEVKFNWYVDGVEVHNAKTKPREEQYNSTYRVVSVLTVLHQDWLNGKEYKCKVSNKALPAPIEKTISKAKGQPREPQVYTLPPCRDELTKNQVSLWCLVKGFYPSDIAVEWESNGQPENNYKTTPPVLDSDGSFFLYSKLTVDKSRWQQGNVFSCSVMHEALHNHYTQKSLSLSPGK

SEQ ID NO: 7 - protein, 366 aa, synthetic construct
APASSSTKKTQLQLEHLLLDLQMILNGINNYKNPKLTRMLTFKFYMPKKATELKHLQCLEEELKPLEEVLNLAGDASIHDLISRINVIVLELKGSETTFMCEYADETATIVEFLNRWITFSQSIIRTLTGGGGSGGGGSDKTHTCPPCPAPEAAGGPSVFLFPPKPKDTLMISRTPEVTCVVVDVSHEDPEVKFNWYVDGVEVHNAKTKPREEQYNSTYRVVSVLTVLHQDWLNGKEYKCKVSNKALPAPIEKTISKAKGQPREPQVYTLPPCRDELTKNQVSLWCLVKGFYPSDIAVEWESNGQPENNYKTTPPVLDSDGSFFLYSKLTVDKSRWQQGNVFSCSVMHEALHNHYTQKSLSLSPGK

SEQ ID NO: 8 - protein, 120 aa, synthetic construct
QVQLVQSGAEVKKPGSSVKVSCKASGGTFSSYAISWVRQAPGQGLEWMGLIIPMFDTAGYAQKFQGRVAITVDESTSTAYMELSSLRSEDTAVYYCARAEHSSTGTFDYWGQGTLVTVSS

SEQ ID NO: 9 - protein, 10 aa, synthetic construct
GGTFSSYAIS

SEQ ID NO: 10 - protein, 17 aa, synthetic construct
LIIPMFDTAGYAQKFQG

SEQ ID NO: 11 - protein, 11 aa, synthetic construct
AEHSSTGTFDY

SEQ ID NO: 12 - protein, 227 aa, synthetic construct
DKTHTCPPCPAPEAAGGPSVFLFPPKPKDTLMISRTPEVTCVVVDVSHEDPEVKFNWYVDGVEVHNAKTKPREEQYNSTYRVVSVLTVLHQDWLNGKEYKCKVSNKALPAPIEKTISKAKGQPREPQVCTLPPSRDELTKNQVSLSCAVKGFYPSDIAVEWESNGQPENNYKTTPPVLDSDGSFFLVSKLTVDKSRWQQGNVFSCSVMHEALHNHYTQKSLSLSPGK

SEQ ID NO: 13 - protein, 330 aa, synthetic construct
ASTKGPSVFPLAPSSKSTSGGTAALGCLVKDYFPEPVTVSWNSGALTSGVHTFPAVLQSSGLYSLSSVVTVPSSSLGTQTYICNVNHKPSNTKVDKKVEPKSCDKTHTCPPCPAPEAAGGPSVFLFPPKPKDTLMISRTPEVTCVVVDVSHEDPEVKFNWYVDGVEVHNAKTKPREEQYNSTYRVVSVLTVLHQDWLNGKEYKCKVSNKALPAPIEKTISKAKGQPREPQVCTLPPSRDELTKNQVSLSCAVKGFYPSDIAVEWESNGQPENNYKTTPPVLDSDGSFFLVSKLTVDKSRWQQGNVFSCSVMHEALHNHYTQKSLSLSPGK

SEQ ID NO: 14 - protein, 450 aa, synthetic construct
QVQLVQSGAEVKKPGSSVKVSCKASGGTFSSYAISWVRQAPGQGLEWMGLIIPMFDTAGYAQKFQGRVAITVDESTSTAYMELSSLRSEDTAVYYCARAEHSSTGTFDYWGQGTLVTVSSASTKGPSVFPLAPSSKSTSGGTAALGCLVKDYFPEPVTVSWNSGALTSGVHTFPAVLQSSGLYSLSSVVTVPSSSLGTQTYICNVNHKPSNTKVDKKVEPKSCDKTHTCPPCPAPEAAGGPSVFLFPPKPKDTLMISRTPEVTCVVVDVSHEDPEVKFNWYVDGVEVHNAKTKPREEQYNSTYRVVSVLTVLHQDWLNGKEYKCKVSNKALPAPIEKTISKAKGQPREPQVCTLPPSRDELTKNQVSLSCAVKGFYPSDIAVEWESNGQPENNYKTTPPVLDSDGSFFLVSKLTVDKSRWQQGNVFSCSVMHEALHNHYTQKSLSLSPGK

SEQ ID NO: 15 - protein, 107 aa, synthetic construct
DIQMTQSPSSVSASVGDRVTITCRASQGISSWLAWYQQKPGKAPKLLISAASSLQSGVPSRFSGSGSGTDFTLTISSLQPEDFATYYCQQANHLPFTFGGGTKVEIK

SEQ ID NO: 16 - protein, 11 aa, synthetic construct
RASQGISSWLA

SEQ ID NO: 17 - protein, 7 aa, synthetic construct
AASSLQS

SEQ ID NO: 18 - protein, 9 aa, synthetic construct
QQANHLPFT

SEQ ID NO: 19 - protein, 107 aa, synthetic construct [sequence omitted]

SEQ ID NO: 20 - protein, 214 aa, synthetic construct
DIQMTQSPSSVSASVGDRVTITCRASQGISSWLAWYQQKPGKAPKLLISAASSLQSGVPSRFSGSGSGTDFTLTISSLQPEDFATYYCQQANHLPFTFGGGTKVEIKRTVAAPSVFIFPPSDEQLKSGTASVVCLLNNFYPREAKVQWKVDNALQSGNSQESVTEQDSKDSTYSLSSTLTLSKADYEKHKVYACEVTHQGLSSPVTKSFNRGEC

SEQ ID NO: 21 - protein, 227 aa, synthetic construct
DKTHTCPPCPAPEAAGGPSVFLFPPKPKDTLMISRTPEVTCVVVDVSHEDPEVKFNWYVDGVEVHNAKTKPREEQYNSTYRVVSVLTVLHQDWLNGKEYKCKVSNKALPAPIEKTISKAKGQPREPQVYTLPPSRDELTKNQVSLTCLVKGFYPSDIAVEWESNGQPENNYKTTPPVLDSDGSFFLYSKLTVDKSRWQQGNVFSCSVMHEALHNHYTQKSLSLSPGK

SEQ ID NO: 22 - protein, 227 aa, synthetic construct
DKTHTCPPCPAPELLGGPSVFLFPPKPKDTLMISRTPEVTCVVVDVSHEDPEVKFNWYVDGVEVHNAKTKPREEQYNSTYRVVSVLTVLHQDWLNGKEYKCKVSNKALPAPIEKTISKAKGQPREPQVYTLPPSRDELTKNQVSLTCLVKGFYPSDIAVEWESNGQPENNYKTTPPVLDSDGSFFLYSKLTVDKSRWQQGNVFSCSVMHEALHNHYTQKSLSLSPGK

SEQ ID NO: 23 - protein, 597 aa, synthetic construct
EVQLLESGGGLVQPGGSLRLSCAASGFSFSSYTMSWVRQAPGKGLEWVATISGGGRDIYYPDSVKGRFTISRDNSKNTLYLQMNSLRAEDTAVYYCVLLTGRVYFALDSWGQGTLVTVSSASTKGPSVFPLAPSSKSTSGGTAALGCLVKDYFPEPVTVSWNSGALTSGVHTFPAVLQSSGLYSLSSVVTVPSSSLGTQTYICNVNHKPSNTKVDKKVEPKSCDKTHTCPPCPAPEAAGGPSVFLFPPKPKDTLMISRTPEVTCVVVDVSHEDPEVKFNWYVDGVEVHNAKTKPREEQYNSTYRVVSVLTVLHQDWLNGKEYKCKVSNKALPAPIEKTISKAKGQPREPQVYTLPPCRDELTKNQVSLWCLVKGFYPSDIAVEWESNGQPENNYKTTPPVLDSDGSFFLYSKLTVDKSRWQQGNVFSCSVMHEALHNHYTQKSLSLSPGGGGGSGGGGSGGGGSAPASSSTKKTQLQLEHLLLDLQMILNGINNYKNPKLTRMLTAKFAMPKKATELKHLQCLEEELKPLEEVLNGAQSKNFHLRPRDLISNINVIVLELKGSETTFMCEYADETATIVEFLNRWITFAQSIISTLT

SEQ ID NO: 24 - protein, 450 aa, synthetic construct
EVQLLESGGGLVQPGGSLRLSCAASGFSFSSYTMSWVRQAPGKGLEWVATISGGGRDIYYPDSVKGRFTISRDNSKNTLYLQMNSLRAEDTAVYYCVLLTGRVYFALDSWGQGTLVTVSSASTKGPSVFPLAPSSKSTSGGTAALGCLVKDYFPEPVTVSWNSGALTSGVHTFPAVLQSSGLYSLSSVVTVPSSSLGTQTYICNVNHKPSNTKVDKKVEPKSCDKTHTCPPCPAPEAAGGPSVFLFPPKPKDTLMISRTPEVTCVVVDVSHEDPEVKFNWYVDGVEVHNAKTKPREEQYNSTYRVVSVLTVLHQDWLNGKEYKCKVSNKALPAPIEKTISKAKGQPREPQVCTLPPSRDELTKNQVSLSCAVKGFYPSDIAVEWESNGQPENNYKTTPPVLDSDGSFFLVSKLTVDKSRWQQGNVFSCSVMHEALHNHYTQKSLSLSPGK

SEQ ID NO: 25 - protein, 218 aa, synthetic construct
DIVMTQSPDSLAVSLGERATINCKASESVDTSDNSFIHWYQQKPGQSPKLLIYRSSTLESGVPDRFSGSGSGTDFTLTISSLQAEDVAVYYCQQNYDVPWTFGQGTKVEIKRTVAAPSVFIFPPSDEQLKSGTASVVCLLNNFYPREAKVQWKVDNALQSGNSQESVTEQDSKDSTYSLSSTLTLSKADYEKHKVYACEVTHQGLSSPVTKSFNRGEC